European Patent Application EP 4 349 328 A1, published April 10, 2024. Title: Low density lipoprotein mimicking solid lipid nanoparticles for drug delivery and uses thereof. Applicant: LIM, duck-soo. The sequence listing filed with the application follows.

SEQUENCE LISTING (16 sequences)

SEQ ID NO: 1 - RNA, 22 nt, Artificial Sequence
  Kras siRNA_#1_sense
ugaauuagcuguaucgucaagg

SEQ ID NO: 2 - RNA, 22 nt, Artificial Sequence
  Kras siRNA_#1_antisense
uugacgauacagcuaauucaua

SEQ ID NO: 3 - RNA, 22 nt, Artificial Sequence
  Kras siRNA_#2_sense
acuguacuccucuugaccugcu

SEQ ID NO: 4 - RNA, 22 nt, Artificial Sequence
  Kras siRNA_#2_antisense
caggucaagaggaguacaguua

SEQ ID NO: 5 - RNA, 22 nt, Artificial Sequence
  Kras siRNA_#3_sense
uauaauggugaauaucuucaaa

SEQ ID NO: 6 - RNA, 22 nt, Artificial Sequence
  Kras siRNA_#3_antisense
ugaagauauucaccauuauaua

SEQ ID NO: 7 - RNA, 23 nt, Artificial Sequence
  Control siRNA_sense
ugugguagcuauacggauadtdt

SEQ ID NO: 8 - RNA, 23 nt, Artificial Sequence
  Control siRNA_antisense
uauccguauagcuaccacadtdt

SEQ ID NO: 9 - DNA, 19 bp, Artificial Sequence
  Human_Kras_Primer_F
aattgtccatctaccatgg

SEQ ID NO: 10 - DNA, 23 bp, Artificial Sequence
  Human_Kras_Primer_R
gaggtcagctgaagcaaatccaa

SEQ ID NO: 11 - DNA, 20 bp, Artificial Sequence
  Human_b-actin_Primer_F
cccaaagttcacaatgtggc

SEQ ID NO: 12 - DNA, 20 bp, Artificial Sequence
  Human_b-actin_Primer_R
agggagaccaaaagccttca

SEQ ID NO: 13 - DNA, 20 bp, Artificial Sequence
  mouse_Kras_Primer_F
tccaacgatcatggacttca

SEQ ID NO: 14 - DNA, 20 bp, Artificial Sequence
  mouse_Kras_Primer_R
caggacttggaggtcttgga

SEQ ID NO: 15 - DNA, 20 bp, Artificial Sequence
  mouse_b-actin_Primer_F
tgttaccaactgggacgaca

SEQ ID NO: 16 - DNA, 16 bp, Artificial Sequence
  mouse_b-actin_Primer_R
aaggaaggctggaaaa